European Patent Specification EP 3 505 532 B1, published July 19, 2023. Title: Chlorotoxin fusion protein with increased skin cell proliferation effect and cosmetic composition for improving skin wrinkle, skin elasticity and anti-aging comprising the same as effective component. Applicant: Nexgen Biotechnologies, Inc. The sequence listing filed with the application follows.

SEQUENCE LISTING (12 sequences)

SEQ ID NO: 1 - DNA, 423 bp, Artificial Sequence
  TRX-CLT
atggtgaagcagatcgagagcaagactgcttttcaggaagccttggacgctgcaggtgataaacttgtagtagttgacttctcagccacgtggtgtgggccttgcaaaatgatcaagcctttctttcattccctctctgaaaagtattccaacgtgatattccttgaagtagatgtggatgactgtcaggatgttgcttcagagtgtgaagtcaaatgcatgccaacattccagttttttaagaagggacaaaaggtgggtgaattttctggagccaataaggaaaagcttgaagccaccattaatgaattagtctgcatgccgtgcttcaccaccgaccaccagatggcgcgtaaatgcgacgactgctgcggtggtaaaggtcgtggtaaatgctacggtccgcagtgcctgtgccgttga

SEQ ID NO: 2 - DNA, 270 bp, Artificial Sequence
  EGF-CLT
atgaactcagactctgagtgcccactgtctcacgacggctactgccttcacgacggagtctgcatgtacatcgaggctttggataagtacgcttgtaattgcgtcgttggttacattggagagcgctgccaataccgtgacttaaaatggtgggagttgcgctgcatgccgtgcttcaccaccgaccaccagatggcgcgtaaatgcgacgactgctgcggtggtaaaggtcgtggtaaatgctacggtccgcagtgcctgtgccgttga

SEQ ID NO: 3 - protein, 140 aa, Artificial Sequence
  TRX-CLT
MVKQIESKTAFQEALDAAGDKLVVVDFSATWCGPCKMIKPFFHSLSEKYSNVIFLEVDVDDCQDVASECEVKCMPTFQFFKKGQKVGEFSGANKEKLEATINELVCMPCFTTDHQMARKCDDCCGGKGRGKCYGPQCLCR

SEQ ID NO: 4 - protein, 89 aa, Artificial Sequence
  EGF-CLT
MNSDSECPLSHDGYCLHDGVCMYIEALDKYACNCVVGYIGERCQYRDLKWWELRCMPCFTTDHQMARKCDDCCGGKGRGKCYGPQCLCR

SEQ ID NO: 5 - DNA, 32 bp, Artificial Sequence
  primer
aaggagatatacatatggtgaagcagatcgag

SEQ ID NO: 6 - DNA, 35 bp, Artificial Sequence
  primer
cgtcacggacacggcagactaattcattaatggtg

SEQ ID NO: 7 - DNA, 37 bp, Artificial Sequence
  primer
caccattaatgaattagtcatgtgcatgccgtgcttc

SEQ ID NO: 8 - DNA, 37 bp, Artificial Sequence
  primer
gaagcacggcatgcacatgactaattcattaatggtg

SEQ ID NO: 9 - DNA, 35 bp, Artificial Sequence
  primer
aaggagatatacatatgaactcagactctgagtgc

SEQ ID NO: 10 - DNA, 34 bp, Artificial Sequence
  primer
ggtggtggtgctcgagacggcacaggcactgcgg

SEQ ID NO: 11 - DNA, 36 bp, Artificial Sequence
  primer
aaatggtgggagttgcgcatgtgcatgccgtgcttc

SEQ ID NO: 12 - DNA, 36 bp, Artificial Sequence
  primer
gaagcacggcatgcacatgcgcaactcccaccattt